European Patent Application EP 4 644 561 A1, published November 5, 2025. Title: OPTICAL, CELL-BASED, HIGH-THROUGHPUT CAPABLE METHOD FOR THE DETERMINATION OF TELOMERE LENGTH AND DYNAMICS IN YEAST. Applicant: HTW Berlin. Application EP. The sequence listing filed with the application follows.

SEQUENCE LISTING (29 sequences)

SEQ ID NO: 1 - DNA, 1044 bp, Renilla reniformis
  source 1..1044: mol_type = genomic DNA
atgactcaattgaacggatctgctagcggaggttctggcgcgccaaccggaaatgtggcttctaaggtttacgacccagaacaaagaaaaaggatgattactggtcctcaatggtgggctagatgcaagcaaatgaatgtcttagattctttcatcaactactatgactcagagaagcacgctgaaaacgcagttatttttttgcacggtaacgctgcatcctcttacttatggaggcacgtcgtacctcatatcgagccagttgccagatgtatcattccagatttgattggtatgggtaagtctggtaaatcaggtaatggctcctatagactattggaccactacaagtacctaactgcttggtttgaattgctaaacttaccaaagaaaatcattttcgtgggacatgattggggttcttgtttggcctttcattattcttacgaacatcaagataagatcaaggctattgttcatgcggaatctgttgtggatgttattgaatcttgggaggattggcctgacattgaagaggatattgctttgttaaagtctgaagagggtgaaaaaatggtgttagaaaataactttttcgttgagactatgttaccatcaaagataatgagaaaattggaacctgaagagtttgctgcttatttggaaccattcaaggaaaaaggcgaggttagaaggcccaccctatcttggcctagagaaatcccattagtcaaaggaggcaagccagatgttgtccagattgttagaaactacaatgcctatttaagggcttctgacgatttacctaagatgttcattgaatccgaccctggtttcttttccaatgccattgtcgaaggtgctaagaaattccctaataccgagtttgttaaggttaagggtttgcacttttctcaagaggatgctccagacgaaatgggtaagtacattaaatccttcgtggaaagggttttgaaaaacgaacagaccgctaacggtgatccgcggagtggaggaaccggtagtggtaacagatcttctaaa

SEQ ID NO: 2 - DNA, 807 bp, synthetic construct
  source 1..807: mol_type = other DNA
atgactcaattgaacggatctgctagcggaggttctggcgcgccaaccggaaatgtgtccaagggtgaagaattgttcactggtgttgtcccaattttggttgaattagatggtgatgttaatgggcacaaattttctgtcagaggagagggtgaaggtgatgcaacaatcggtaagttgaccttgaaagtcatttgcactactggtaaactacctgttccttggcctaccttggtcactactgttggttatggtgttcaatgctttgctagatacccagatcacatgaagcaacatgacttttacaagagtgccatgccagaaggttatgttcaggaaagaactatctccttcaaagatgacggtaagtacaagactcgtgctgaagtcaagtttgaaggtgataccttggttaatagaatcgagttaaagggtattgattttaaggaagatggtaacattttaggtcacaaattggcttacaactttaactctcacaatgtttacatcactgctgacaagcaaaagaacggtatcaaggctaacttcaaaattagacacaacattgaggatggtggtgttcaactagctgaccattatcaacaaaatactccaatcggcgatggccctgtccttttaccagacaaccattacctgtcctaccaatctcgtgtttacaaagatccaaacgaaaagagagaccacatggctgttattgagtttatgactgctgctggaattactcatggcatggatgaactaccgcggagtggaggaaccggtagtggtaacagatcttctaaataa

SEQ ID NO: 3 - DNA, 2232 bp, synthetic construct
  source 1..2232: mol_type = other DNA
atggagcatgtagattccgattttgcacctataaggagatcgaaaaaggttgttgacagtgacaagattgtgaaagcaataagcgatgatttggagcaaaaaaattttactgtactgagaaagttgaaccttgttccaattaaaaaaagtgttagcagcccaaaggtgtgtaagccgagtccagttaaggagcgagtggaccatgttttctaccagaagttcaaatcaatggccttgcaagagctaggcaccaattatttgtcaataagctacgttccgagcttaagtaagtttctttcaaaaaatcttaggagtatgaaaaattgtatcgttttcttcgacaaagttgaacatatacaccaatatgctggtatcgaccgtgcagtttcagaaacactgtctttagtcgatataaatgtcgtaattatagaaatgaatgactacttaatgaaagagggtattcaatcaagcaaatcaaaagaatgtatcgagtcaatggggcaggcttcatatagcggacaactagatttcgaagctagtgaaaaaccttcaaatcacacgtctgacctaatgatgatggttatgaggaaaataaataatgacgaaagtatcgatcatattgtctacttcaaattcgaacaattagataaattatctacttcaactataatagaaccttcgaagcttaccgaatttatcaatgttttatcggtacttgaaaaaagtaataacattgcatttaaggtcctcatttattcaaataacgttagcatttcgtctctcctatcgacatccctcaaaaagaaactcaacacaaaatatactgtgtttgagatgccgatattaacatgcgctcaagaacaagaatatttgaaaaaaatgataaagtttacctttgattccggaagcaagttattacagtcttacaactcgcttgtcacatgccagttgaataataaagaatccaacttagcaatctttttcgaatttttgaaggtctttccgcacccttttacctatttgtttaacgcttacactgagattatagtccagagtagaacttttgatgaattgttggataagatcagaaacagactgacaataaaaaattacccacatagtgcttataactttaagaaaaaccagcgtcttccacttaagttaactcgaaaagtacatgatagaatgactcaattgaacggatctgctagcggaggttctggcgcgccaaccggaaatgtggcttctaaggtttacgacccagaacaaagaaaaaggatgattactggtcctcaatggtgggctagatgcaagcaaatgaatgtcttagattctttcatcaactactatgactcagagaagcacgctgaaaacgcagttatttttttgcacggtaacgctgcatcctcttacttatggaggcacgtcgtacctcatatcgagccagttgccagatgtatcattccagatttgattggtatgggtaagtctggtaaatcaggtaatggctcctatagactattggaccactacaagtacctaactgcttggtttgaattgctaaacttaccaaagaaaatcattttcgtgggacatgattggggttcttgtttggcctttcattattcttacgaacatcaagataagatcaaggctattgttcatgcggaatctgttgtggatgttattgaatcttgggaggattggcctgacattgaagaggatattgctttgttaaagtctgaagagggtgaaaaaatggtgttagaaaataactttttcgttgagactatgttaccatcaaagataatgagaaaattggaacctgaagagtttgctgcttatttggaaccattcaaggaaaaaggcgaggttagaaggcccaccctatcttggcctagagaaatcccattagtcaaaggaggcaagccagatgttgtccagattgttagaaactacaatgcctatttaagggcttctgacgatttacctaagatgttcattgaatccgaccctggtttcttttccaatgccattgtcgaaggtgctaagaaattccctaataccgagtttgttaaggttaagggtttgcacttttctcaagaggatgctccagacgaaatgggtaagtacattaaatccttcgtggaaagggttttgaaaaacgaacagaccgctaacggtgatccgcggagtggaggaaccggtagtggtaacagatcttctaaataa

SEQ ID NO: 4 - DNA, 3288 bp, synthetic construct
  source 1..3288: mol_type = other DNA
atgtctagtccagatgattttgaaactgcaccagcagaatatgttgatgcattggatccgagtatggtcgttgttgacagtggttctgctgcagtcacagcgccatcggattcagccgctgaggtaaaagctaatcaaaacgaagaaaacactggtgctactgctgctgaaactagtgagaaagtggatcagacggaggtcgaaaagaaagatgatgatgataccactgaagtcggtgtaacaactaccacgccttccattgctgatactgctgctaccgctaacattgcttcgacatcaggtgcatctgttactgaacctactactgatgacaccgctgctgatgagaaaaaggaacaagtaagtggtcctcctctgtcaaatatgaaattctatcttaatcgcgacgcggatgcgcatgactctttaaatgatattgatcaattagcgcgtctgattagagcaaacggtggtgaagtgctagactccaagccaagagaatcaaaagagaatgttttcatcgtgtcaccctataatcataccaatttaccaacggtaactccgacttatattaaggcatgttgtcaaagcaactcgctactgaacatggaaaattatttagtaccatacgataactttagagaagttgtcgatagtaggttgcaggaggaatcgcattctaatggtgtagataatagcaatagcaatagcgataacaaggattctatcaggcccaaaacagaaataatctctacgaatactaatggcgctacggaagactcaaccagcgaaaaagttatggtagacgctgaacaacaagctagattacaagagcaagctcagctccttcgtcaacatgtaagcagcaccgcatcaatcacaagcggagggcacaatgacttggtccagatcgaacaacctcaaaaagatacctccaataataataatagcaacgtcaacgacgaagacaatgatcttttgacacaggacaacaaccctcaaacagcagatgaggggaatgcatcttttcaagcacaaaggtccatgatttcgagaggcgctttgccctcccacaataaagcttcttttacagatgaggaagatgagtttattttggatgttgtgagaaaaaatccaaccaggcgtacaacacatactctttacgatgaaatatcccattatgtgcctaaccacacgggtaattctattaggcaccgatttagagtctatctttccaaaagactagagtacgtttatgaggttgacaagtttggtaaattggttagagacgacgatggaaatctgataaagactaaagttttgccaccatcaattaaaaggaaattttcagcagatgaagattacactttggcaatcgcggtcaagaagcagttttatcgtgatttgtttcaaatcgaccctgatactggaagatcacttatcacagatgaggatacacccactgctatagcgaggaggaatatgacaatggatccaaatcatgtgccagggagtgaacccaactttgcagcttacagaacccaaagccgtaggggaccgattgcacgagaatttttcaagcattttgccgaagagcatgcagcacatactgagaatgcttggagagataggtttaggaagtttcttctcgcttacggcattgatgattatattagttattatgaagctgaaaaagctcagaatagagagccggaaccgatgaagaacctcaccaatagacccaagaggcctggcgttcccactcctggcaattataactctgccgccaagagggcaagaaattatagttctcaaagaaatgttcagcctactgccaatgcagcgtccgctaatgctgctgccgctgctgctgccgctgcttccaactcttacgctataccagaaaacgaattactggacgaagataccatgaatttcatttccagtttaaagaatgatctatccaatatttcaaatagtttgccctttgagtatccacacgagattgcggaagctataagaagcgatttttcgaatgaagatatatatgataatattgatcctgataccataagctttccaccaaaaattgcaacaacagatcttttcctgccattgttctttcattttggcagtacgagacaatttatggataaacttcatgaagttatttcaggagattatgagccatcacaggctgaaaaactggtacaggatctttgcgatgaaactggtatacgtaaaaatttcagtacgagcatattgacgtgtttatccggggatctgatggtctttcctcgctatttcttgaacatgtttaaggacaatgttaatcctcctcccaacgttcctggtatttggacacatgatgacgacgaatcgctaaaaagcaatgatcaagaacaaataaggaaactggttaaaaagcatggaactggtagaatggaaatgaggaaaagattttttgagaaggacctgttaatgactcaattgaacggatctgctagcggaggttctggcgcgccaaccggaaatgtgtccaagggtgaagaattgttcactggtgttgtcccaattttggttgaattagatggtgatgttaatgggcacaaattttctgtcagaggagagggtgaaggtgatgcaacaatcggtaagttgaccttgaaagtcatttgcactactggtaaactacctgttccttggcctaccttggtcactactgttggttatggtgttcaatgctttgctagatacccagatcacatgaagcaacatgacttttacaagagtgccatgccagaaggttatgttcaggaaagaactatctccttcaaagatgacggtaagtacaagactcgtgctgaagtcaagtttgaaggtgataccttggttaatagaatcgagttaaagggtattgattttaaggaagatggtaacattttaggtcacaaattggcttacaactttaactctcacaatgtttacatcactgctgacaagcaaaagaacggtatcaaggctaacttcaaaattagacacaacattgaggatggtggtgttcaactagctgaccattatcaacaaaatactccaatcggcgatggccctgtccttttaccagacaaccattacctgtcctaccaatctcgtgtttacaaagatccaaacgaaaagagagaccacatggctgttattgagtttatgactgctgctggaattactcatggcatggatgaactaccgcggagtggaggaaccggtagtggtaacagatcttctaaataa

SEQ ID NO: 5 - DNA, 20 bp, synthetic construct
  source 1..20: mol_type = other DNA
gaatgaaaaaaagtaaagca

SEQ ID NO: 6 - DNA, 20 bp, synthetic construct
  source 1..20: mol_type = other DNA
gctattggtgattcgcattt

SEQ ID NO: 7 - DNA, 20 bp, synthetic construct
  source 1..20: mol_type = other DNA
ttatttcactgattcacgtt

SEQ ID NO: 8 - DNA, 20 bp, synthetic construct
  source 1..20: mol_type = other DNA
aattcttacaatgattaagg

SEQ ID NO: 9 - DNA, 20 bp, synthetic construct
  source 1..20: mol_type = other DNA
tctccttataggtgcaaaat

SEQ ID NO: 10 - DNA, 20 bp, synthetic construct
  source 1..20: mol_type = other DNA
cgatccgaagctacttatgc

SEQ ID NO: 11 - DNA, 20 bp, synthetic construct
  source 1..20: mol_type = other DNA
gttgtccgctatatgaagcc

SEQ ID NO: 12 - DNA, 47 bp, synthetic construct
  source 1..47: mol_type = other DNA
cgaacgtggttagtatatagagacaatgactcaattgaacggatctg

SEQ ID NO: 13 - DNA, 51 bp, synthetic construct
  source 1..51: mol_type = other DNA
gcaaagtcggaatctacatgctccattttagaagatctgttaccactaccg

SEQ ID NO: 14 - DNA, 47 bp, synthetic construct
  source 1..47: mol_type = other DNA
cagatccgttcaattgagtcattgtctctatatactaaccacgttcg

SEQ ID NO: 15 - DNA, 51 bp, synthetic construct
  source 1..51: mol_type = other DNA
cggtagtggtaacagatcttctaaaatggagcatgtagattccgactttgc

SEQ ID NO: 16 - DNA, 19 bp, synthetic construct
  source 1..19: mol_type = other DNA
ctaacggtgatccgcggag

SEQ ID NO: 17 - DNA, 25 bp, synthetic construct
  source 1..25: mol_type = other DNA
ccatcatcattaggtcagacgtgtg

SEQ ID NO: 18 - DNA, 20 bp, synthetic construct
  source 1..20: mol_type = other DNA
caatagacccaagaggcctg

SEQ ID NO: 19 - DNA, 23 bp, synthetic construct
  source 1..23: mol_type = other DNA
cttccagcaaatctaacagcatc

SEQ ID NO: 20 - DNA, 50 bp, synthetic construct
  source 1..50: mol_type = other DNA
gaaaagattttttgagaaggacctgttaatgactcaattgaacggatctg

SEQ ID NO: 21 - DNA, 49 bp, synthetic construct
  source 1..49: mol_type = other DNA
gctaatgggattctataaaactgttccggtaccattaccctgttatccc

SEQ ID NO: 22 - DNA, 50 bp, synthetic construct
  source 1..50: mol_type = other DNA
cagatccgttcaattgagtcattaacaggtccttctcaaaaaatcttttc

SEQ ID NO: 23 - DNA, 49 bp, synthetic construct
  source 1..49: mol_type = other DNA
gggataacagggtaatggtaccggaacagttttatagaatcccattagc

SEQ ID NO: 24 - DNA, 23 bp, synthetic construct
  source 1..23: mol_type = other DNA
cttattgaccacacctctaccgg

SEQ ID NO: 25 - DNA, 26 bp, synthetic construct
  source 1..26: mol_type = other DNA
ctgttaatttctttttagacccacca

SEQ ID NO: 26 - DNA, 120 bp, synthetic construct
  source 1..120: mol_type = other DNA
gaagccgattttctattatcccgttctgataatcgatttttagcggattattaactttcttaaccataactaacacgccctcatgaatattatcctctaagataaaacacagatcgacag

SEQ ID NO: 27 - DNA, 120 bp, synthetic construct
  source 1..120: mol_type = other DNA
aagtgaccacattttaaattttctttgtaagtactgttggtctgtagatcaatgtcaagcttgtcttgaatgaactcgaataagattttcatgattgattcttttgaagagaagcaaggc

SEQ ID NO: 28 - DNA, 23 bp, synthetic construct
  source 1..23: mol_type = other DNA
tctaagataaaacacagatcgac

SEQ ID NO: 29 - DNA, 20 bp, synthetic construct
  source 1..20: mol_type = other DNA
ccaggaaggcatggtaatgc